European Patent Specification EP 3 871 685 B1, published August 30, 2023. Title: an anti-obesity agent, an agent for improving frequent urination, and an agent for regulating autonomic nerve activity. Applicant: ASAHI GROUP HOLDINGS, LTD. The sequence listing filed with the application follows.

SEQUENCE LISTING (1 sequence)

SEQ ID NO: 1 - protein, 19 aa, artificial
  functional peptide
NIPPLTQTPVVVPPFLQPE